European Patent Specification EP 3 645 034 B1, published August 30, 2023. Title: 21-day Dosing Regimen for Fusion Proteins Comprising Factor IX and Human Albumin for Prophlylactic Treatment of Hemophilia and Methods Thereof. Applicant: CSL Behring Recombinant Facility AG. The sequence listing filed with the application follows.

SEQUENCE LISTING (4 sequences)

SEQ ID NO: 1 - protein, 1018 aa, Artificial Sequence
  Fusion Protein
  FIX (1)..(415)
  Linker (416)..(433)
  Human Albumin (434)..(1018)
YNSGKLEEFVQGNLERECMEEKCSFEEAREVFENTERTTEFWKQYVDGDQCESNPCLNGGSCKDDINSYECWCPFGFEGKNCELDVTCNIKNGRCEQFCKNSADNKVVCSCTEGYRLAENQKSCEPAVPFPCGRVSVSQTSKLTRAETVFPDVDYVNSTEAETILDNITQSTQSFNDFTRVVGGEDAKPGQFPWQVVLNGKVDAFCGGSIVNEKWIVTAAHCVETGVKITVVAGEHNIEETEHTEQKRNVIRIIPHHNYNAAINKYNHDIALLELDEPLVLNSYVTPICIADKEYTNIFLKFGSGYVSGWGRVFHKGRSALVLQYLRVPLVDRATCLRSTKFTIYNNMFCAGFHEGGRDSCQGDSGGPHVTEVEGTSFLTGIISWGEECAMKGKYGIYTKVSRYVNWIKEKTKLTPVSQTSKLTRAETVFPDVDAHKSEVAHRFKDLGEENFKALVLIAFAQYLQQCPFEDHVKLVNEVTEFAKTCVADESAENCDKSLHTLFGDKLCTVATLRETYGEMADCCAKQEPERNECFLQHKDDNPNLPRLVRPEVDVMCTAFHDNEETFLKKYLYEIARRHPYFYAPELLFFAKRYKAAFTECCQAADKAACLLPKLDELRDEGKASSAKQRLKCASLQKFGERAFKAWAVARLSQRFPKAEFAEVSKLVTDLTKVHTECCHGDLLECADDRADLAKYICENQDSISSKLKECCEKPLLEKSHCIAEVENDEMPADLPSLAADFVESKDVCKNYAEAKDVFLGMFLYEYARRHPDYSVVLLLRLAKTYETTLEKCCAAADPHECYAKVFDEFKPLVEEPQNLIKQNCELFEQLGEYKFQNALLVRYTKKVPQVSTPTLVEVSRNLGKVGSKCCKHPEAKRMPCAEDYLSVVLNQLCVLHEKTPVSDRVTKCCTESLVNRRPCFSALEVDETYVPKEFNAETFTFHADICTLSEKERQIKKQTALVELVKHKPKATKEQLKAVMDDFAAFVEKCCKADDKETCFAEEGKKLVAASQAALGL

SEQ ID NO: 2 - protein, 18 aa, Artificial Sequence
  Linker
PVSQTSKLTRAETVFPDV

SEQ ID NO: 3 - protein, 19 aa, Artificial Sequence
  Linker
PSVSQTSKLTRAETVFPDV

SEQ ID NO: 4 - protein, 7 aa, Artificial Sequence
  Linker
GGGGGGV